European Patent Application EP 4 596 693 A1, published August 6, 2025. Title: 用于抑制TMPRSS6基因表达的siRNA或其盐、药物及其应用. Applicant: 广州必贝特医药股份有限公司. Application CN. The sequence listing filed with the application follows.

SEQUENCE LISTING (188 sequences)

SEQ ID NO: 1 - RNA, 19 nt, synthetic construct
  source 1..19: mol_type = other RNA
tcacctgcttcttctggtt

SEQ ID NO: 2 - RNA, 19 nt, synthetic construct
  source 1..19: mol_type = other RNA
aaccagaagaagcaggtga

SEQ ID NO: 3 - RNA, 21 nt, synthetic construct
  source 1..21: mol_type = other RNA
gccaaagcccagaagatgcta

SEQ ID NO: 4 - RNA, 23 nt, synthetic construct
  source 1..23: mol_type = other RNA
tagcatcttctgggctttggcgg

SEQ ID NO: 5 - RNA, 21 nt, synthetic construct
  source 1..21: mol_type = other RNA
tcctttggggagggaccccta

SEQ ID NO: 6 - RNA, 23 nt, synthetic construct
  source 1..23: mol_type = other RNA
taggggtccctccccaaaggaat

SEQ ID NO: 7 - RNA, 21 nt, synthetic construct
  source 1..21: mol_type = other RNA
gtgatcctggaagccagtgta

SEQ ID NO: 8 - RNA, 23 nt, synthetic construct
  source 1..23: mol_type = other RNA
tacactggcttccaggatcacta

SEQ ID NO: 9 - RNA, 21 nt, synthetic construct
  source 1..21: mol_type = other RNA
tgatcctggaagccagtgtga

SEQ ID NO: 10 - RNA, 23 nt, synthetic construct
  source 1..23: mol_type = other RNA
tcacactggcttccaggatcacc

SEQ ID NO: 11 - RNA, 21 nt, synthetic construct
  source 1..21: mol_type = other RNA
gatcctggaagccagtgtgaa

SEQ ID NO: 12 - RNA, 23 nt, synthetic construct
  source 1..23: mol_type = other RNA
ttcacactggcttccaggatcac

SEQ ID NO: 13 - RNA, 21 nt, synthetic construct
  source 1..21: mol_type = other RNA
ccctctctggactacggctta

SEQ ID NO: 14 - RNA, 23 nt, synthetic construct
  source 1..23: mol_type = other RNA
taagccgtagtccagagagggca

SEQ ID NO: 15 - RNA, 21 nt, synthetic construct
  source 1..21: mol_type = other RNA
gatccagaacaggaggctgta

SEQ ID NO: 16 - RNA, 23 nt, synthetic construct
  source 1..23: mol_type = other RNA
tacagcctcctgttctggatcgt

SEQ ID NO: 17 - RNA, 21 nt, synthetic construct
  source 1..21: mol_type = other RNA
atccagaacaggaggctgtgt

SEQ ID NO: 18 - RNA, 23 nt, synthetic construct
  source 1..23: mol_type = other RNA
acacagcctcctgttctggatcg

SEQ ID NO: 19 - RNA, 21 nt, synthetic construct
  source 1..21: mol_type = other RNA
tccagaacaggaggctgtgta

SEQ ID NO: 20 - RNA, 23 nt, synthetic construct
  source 1..23: mol_type = other RNA
tacacagcctcctgttctggatc

SEQ ID NO: 21 - RNA, 21 nt, synthetic construct
  source 1..21: mol_type = other RNA
ccagaacaggaggctgtgtga

SEQ ID NO: 22 - RNA, 23 nt, synthetic construct
  source 1..23: mol_type = other RNA
tcacacagcctcctgttctggat

SEQ ID NO: 23 - RNA, 21 nt, synthetic construct
  source 1..21: mol_type = other RNA
cagaacaggaggctgtgtgga

SEQ ID NO: 24 - RNA, 23 nt, synthetic construct
  source 1..23: mol_type = other RNA
tccacacagcctcctgttctgga

SEQ ID NO: 25 - RNA, 21 nt, synthetic construct
  source 1..21: mol_type = other RNA
gaacaggaggctgtgtggctt

SEQ ID NO: 26 - RNA, 23 nt, synthetic construct
  source 1..23: mol_type = other RNA
aagccacacagcctcctgttctg

SEQ ID NO: 27 - RNA, 21 nt, synthetic construct
  source 1..21: mol_type = other RNA
tcaccatcaacttcacctcca

SEQ ID NO: 28 - RNA, 23 nt, synthetic construct
  source 1..23: mol_type = other RNA
tggaggtgaagttgatggtgatc

SEQ ID NO: 29 - RNA, 21 nt, synthetic construct
  source 1..21: mol_type = other RNA
caccatcaacttcacctccca

SEQ ID NO: 30 - RNA, 23 nt, synthetic construct
  source 1..23: mol_type = other RNA
tgggaggtgaagttgatggtgat

SEQ ID NO: 31 - RNA, 21 nt, synthetic construct
  source 1..21: mol_type = other RNA
accatcaacttcacctcccaa

SEQ ID NO: 32 - RNA, 23 nt, synthetic construct
  source 1..23: mol_type = other RNA
ttgggaggtgaagttgatggtga

SEQ ID NO: 33 - RNA, 21 nt, synthetic construct
  source 1..21: mol_type = other RNA
ccatcaacttcacctcccaga

SEQ ID NO: 34 - RNA, 23 nt, synthetic construct
  source 1..23: mol_type = other RNA
tctgggaggtgaagttgatggtg

SEQ ID NO: 35 - RNA, 21 nt, synthetic construct
  source 1..21: mol_type = other RNA
catcaacttcacctcccagat

SEQ ID NO: 36 - RNA, 23 nt, synthetic construct
  source 1..23: mol_type = other RNA
atctgggaggtgaagttgatggt

SEQ ID NO: 37 - RNA, 21 nt, synthetic construct
  source 1..21: mol_type = other RNA
atcaacttcacctcccagata

SEQ ID NO: 38 - RNA, 23 nt, synthetic construct
  source 1..23: mol_type = other RNA
tatctgggaggtgaagttgatgg

SEQ ID NO: 39 - RNA, 21 nt, synthetic construct
  source 1..21: mol_type = other RNA
tcaacttcacctcccagatct

SEQ ID NO: 40 - RNA, 23 nt, synthetic construct
  source 1..23: mol_type = other RNA
agatctgggaggtgaagttgatg

SEQ ID NO: 41 - RNA, 21 nt, synthetic construct
  source 1..21: mol_type = other RNA
caacttcacctcccagatcta

SEQ ID NO: 42 - RNA, 23 nt, synthetic construct
  source 1..23: mol_type = other RNA
tagatctgggaggtgaagttgat

SEQ ID NO: 43 - RNA, 21 nt, synthetic construct
  source 1..21: mol_type = other RNA
aacttcacctcccagatctca

SEQ ID NO: 44 - RNA, 23 nt, synthetic construct
  source 1..23: mol_type = other RNA
tgagatctgggaggtgaagttga

SEQ ID NO: 45 - RNA, 21 nt, synthetic construct
  source 1..21: mol_type = other RNA
acttcacctcccagatctcca

SEQ ID NO: 46 - RNA, 23 nt, synthetic construct
  source 1..23: mol_type = other RNA
tggagatctgggaggtgaagttg

SEQ ID NO: 47 - RNA, 21 nt, synthetic construct
  source 1..21: mol_type = other RNA
cttcacctcccagatctccct

SEQ ID NO: 48 - RNA, 23 nt, synthetic construct
  source 1..23: mol_type = other RNA
agggagatctgggaggtgaagtt

SEQ ID NO: 49 - RNA, 21 nt, synthetic construct
  source 1..21: mol_type = other RNA
ttcacctcccagatctcccta

SEQ ID NO: 50 - RNA, 23 nt, synthetic construct
  source 1..23: mol_type = other RNA
tagggagatctgggaggtgaagt

SEQ ID NO: 51 - RNA, 21 nt, synthetic construct
  source 1..21: mol_type = other RNA
tcacctcccagatctccctca

SEQ ID NO: 52 - RNA, 23 nt, synthetic construct
  source 1..23: mol_type = other RNA
tgagggagatctgggaggtgaag

SEQ ID NO: 53 - RNA, 21 nt, synthetic construct
  source 1..21: mol_type = other RNA
cacctcccagatctccctcaa

SEQ ID NO: 54 - RNA, 23 nt, synthetic construct
  source 1..23: mol_type = other RNA
ttgagggagatctgggaggtgaa

SEQ ID NO: 55 - RNA, 21 nt, synthetic construct
  source 1..21: mol_type = other RNA
ccagtgtgaggaccggagcta

SEQ ID NO: 56 - RNA, 23 nt, synthetic construct
  source 1..23: mol_type = other RNA
tagctccggtcctcacactggaa

SEQ ID NO: 57 - RNA, 21 nt, synthetic construct
  source 1..21: mol_type = other RNA
cactgtgactgtggcctccaa

SEQ ID NO: 58 - RNA, 23 nt, synthetic construct
  source 1..23: mol_type = other RNA
ttggaggccacagtcacagtgct

SEQ ID NO: 59 - RNA, 21 nt, synthetic construct
  source 1..21: mol_type = other RNA
ttcggggtcgacacatctgta

SEQ ID NO: 60 - RNA, 23 nt, synthetic construct
  source 1..23: mol_type = other RNA
tacagatgtgtcgaccccgaacc

SEQ ID NO: 61 - RNA, 21 nt, synthetic construct
  source 1..21: mol_type = other RNA
tcggggtcgacacatctgtga

SEQ ID NO: 62 - RNA, 23 nt, synthetic construct
  source 1..23: mol_type = other RNA
tcacagatgtgtcgaccccgaac

SEQ ID NO: 63 - RNA, 21 nt, synthetic construct
  source 1..21: mol_type = other RNA
cggggtcgacacatctgtgga

SEQ ID NO: 64 - RNA, 23 nt, synthetic construct
  source 1..23: mol_type = other RNA
tccacagatgtgtcgaccccgaa

SEQ ID NO: 65 - RNA, 21 nt, synthetic construct
  source 1..21: mol_type = other RNA
ccaggaggacagcatggccta

SEQ ID NO: 66 - RNA, 23 nt, synthetic construct
  source 1..23: mol_type = other RNA
taggccatgctgtcctcctggaa

SEQ ID NO: 67 - RNA, 21 nt, synthetic construct
  source 1..21: mol_type = other RNA
cttccaggaggacagcatgga

SEQ ID NO: 68 - RNA, 23 nt, synthetic construct
  source 1..23: mol_type = other RNA
tccatgctgtcctcctggaagca

SEQ ID NO: 69 - RNA, 21 nt, synthetic construct
  source 1..21: mol_type = other RNA
gcttccaggaggacagcatga

SEQ ID NO: 70 - RNA, 23 nt, synthetic construct
  source 1..23: mol_type = other RNA
tcatgctgtcctcctggaagcag

SEQ ID NO: 71 - RNA, 21 nt, synthetic construct
  source 1..21: mol_type = other RNA
tgcttccaggaggacagcata

SEQ ID NO: 72 - RNA, 23 nt, synthetic construct
  source 1..23: mol_type = other RNA
tatgctgtcctcctggaagcagt

SEQ ID NO: 73 - RNA, 21 nt, synthetic construct
  source 1..21: mol_type = other RNA
ctgcttccaggaggacagcat

SEQ ID NO: 74 - RNA, 23 nt, synthetic construct
  source 1..23: mol_type = other RNA
atgctgtcctcctggaagcagtg

SEQ ID NO: 75 - RNA, 21 nt, synthetic construct
  source 1..21: mol_type = other RNA
gtgtccttcaaggtgagccga

SEQ ID NO: 76 - RNA, 23 nt, synthetic construct
  source 1..23: mol_type = other RNA
tcggctcaccttgaaggacacct

SEQ ID NO: 77 - RNA, 21 nt, synthetic construct
  source 1..21: mol_type = other RNA
ggtgtccttcaaggtgagcca

SEQ ID NO: 78 - RNA, 23 nt, synthetic construct
  source 1..23: mol_type = other RNA
tggctcaccttgaaggacacctc

SEQ ID NO: 79 - RNA, 21 nt, synthetic construct
  source 1..21: mol_type = other RNA
aggtgtccttcaaggtgagca

SEQ ID NO: 80 - RNA, 23 nt, synthetic construct
  source 1..23: mol_type = other RNA
tgctcaccttgaaggacacctct

SEQ ID NO: 81 - RNA, 21 nt, synthetic construct
  source 1..21: mol_type = other RNA
agccatgactacgacgtggca

SEQ ID NO: 82 - RNA, 23 nt, synthetic construct
  source 1..23: mol_type = other RNA
tgccacgtcgtagtcatggctgt

SEQ ID NO: 83 - RNA, 21 nt, synthetic construct
  source 1..21: mol_type = other RNA
cagccatgactacgacgtgga

SEQ ID NO: 84 - RNA, 23 nt, synthetic construct
  source 1..23: mol_type = other RNA
tccacgtcgtagtcatggctgtc

SEQ ID NO: 85 - RNA, 21 nt, synthetic construct
  source 1..21: mol_type = other RNA
acagccatgactacgacgtga

SEQ ID NO: 86 - RNA, 23 nt, synthetic construct
  source 1..23: mol_type = other RNA
tcacgtcgtagtcatggctgtcc

SEQ ID NO: 87 - RNA, 21 nt, synthetic construct
  source 1..21: mol_type = other RNA
gacagccatgactacgacgta

SEQ ID NO: 88 - RNA, 23 nt, synthetic construct
  source 1..23: mol_type = other RNA
tacgtcgtagtcatggctgtcct

SEQ ID NO: 89 - RNA, 21 nt, synthetic construct
  source 1..21: mol_type = other RNA
ggacagccatgactacgacgt

SEQ ID NO: 90 - RNA, 23 nt, synthetic construct
  source 1..23: mol_type = other RNA
acgtcgtagtcatggctgtcctc

SEQ ID NO: 91 - RNA, 21 nt, synthetic construct
  source 1..21: mol_type = other RNA
aggacagccatgactacgaca

SEQ ID NO: 92 - RNA, 23 nt, synthetic construct
  source 1..23: mol_type = other RNA
tgtcgtagtcatggctgtcctct

SEQ ID NO: 93 - RNA, 21 nt, synthetic construct
  source 1..21: mol_type = other RNA
gaggacagccatgactacgaa

SEQ ID NO: 94 - RNA, 23 nt, synthetic construct
  source 1..23: mol_type = other RNA
ttcgtagtcatggctgtcctctt

SEQ ID NO: 95 - RNA, 21 nt, synthetic construct
  source 1..21: mol_type = other RNA
cgcctgggaacttactacaat

SEQ ID NO: 96 - RNA, 23 nt, synthetic construct
  source 1..23: mol_type = other RNA
attgtagtaagttcccaggcggg

SEQ ID NO: 97 - RNA, 21 nt, synthetic construct
  source 1..21: mol_type = other RNA
gcctgggaacttactacaact

SEQ ID NO: 98 - RNA, 23 nt, synthetic construct
  source 1..23: mol_type = other RNA
agttgtagtaagttcccaggcgg

SEQ ID NO: 99 - RNA, 21 nt, synthetic construct
  source 1..21: mol_type = other RNA
cctgggaacttactacaacta

SEQ ID NO: 100 - RNA, 23 nt, synthetic construct
  source 1..23: mol_type = other RNA
tagttgtagtaagttcccaggcg

SEQ ID NO: 101 - RNA, 21 nt, synthetic construct
  source 1..21: mol_type = other RNA
ctgggaacttactacaactca

SEQ ID NO: 102 - RNA, 23 nt, synthetic construct
  source 1..23: mol_type = other RNA
tgagttgtagtaagttcccaggc

SEQ ID NO: 103 - RNA, 21 nt, synthetic construct
  source 1..21: mol_type = other RNA
tgggaacttactacaactcca

SEQ ID NO: 104 - RNA, 23 nt, synthetic construct
  source 1..23: mol_type = other RNA
tggagttgtagtaagttcccagg

SEQ ID NO: 105 - RNA, 21 nt, synthetic construct
  source 1..21: mol_type = other RNA
gggaacttactacaactccaa

SEQ ID NO: 106 - RNA, 23 nt, synthetic construct
  source 1..23: mol_type = other RNA
ttggagttgtagtaagttcccag

SEQ ID NO: 107 - RNA, 21 nt, synthetic construct
  source 1..21: mol_type = other RNA
ggaacttactacaactccaga

SEQ ID NO: 108 - RNA, 23 nt, synthetic construct
  source 1..23: mol_type = other RNA
tctggagttgtagtaagttccca

SEQ ID NO: 109 - RNA, 21 nt, synthetic construct
  source 1..21: mol_type = other RNA
gaacttactacaactccagct

SEQ ID NO: 110 - RNA, 23 nt, synthetic construct
  source 1..23: mol_type = other RNA
agctggagttgtagtaagttccc

SEQ ID NO: 111 - RNA, 21 nt, synthetic construct
  source 1..21: mol_type = other RNA
aacttactacaactccagcta

SEQ ID NO: 112 - RNA, 23 nt, synthetic construct
  source 1..23: mol_type = other RNA
tagctggagttgtagtaagttcc

SEQ ID NO: 113 - RNA, 21 nt, synthetic construct
  source 1..21: mol_type = other RNA
acttactacaactccagctca

SEQ ID NO: 114 - RNA, 23 nt, synthetic construct
  source 1..23: mol_type = other RNA
tgagctggagttgtagtaagttc

SEQ ID NO: 115 - RNA, 21 nt, synthetic construct
  source 1..21: mol_type = other RNA
cttactacaactccagctcca

SEQ ID NO: 116 - RNA, 23 nt, synthetic construct
  source 1..23: mol_type = other RNA
tggagctggagttgtagtaagtt

SEQ ID NO: 117 - RNA, 21 nt, synthetic construct
  source 1..21: mol_type = other RNA
ttactacaactccagctccgt

SEQ ID NO: 118 - RNA, 23 nt, synthetic construct
  source 1..23: mol_type = other RNA
acggagctggagttgtagtaagt

SEQ ID NO: 119 - RNA, 21 nt, synthetic construct
  source 1..21: mol_type = other RNA
tactacaactccagctccgta

SEQ ID NO: 120 - RNA, 23 nt, synthetic construct
  source 1..23: mol_type = other RNA
tacggagctggagttgtagtaag

SEQ ID NO: 121 - RNA, 21 nt, synthetic construct
  source 1..21: mol_type = other RNA
actacaactccagctccgtct

SEQ ID NO: 122 - RNA, 23 nt, synthetic construct
  source 1..23: mol_type = other RNA
agacggagctggagttgtagtaa

SEQ ID NO: 123 - RNA, 21 nt, synthetic construct
  source 1..21: mol_type = other RNA
ctacaactccagctccgtcta

SEQ ID NO: 124 - RNA, 23 nt, synthetic construct
  source 1..23: mol_type = other RNA
tagacggagctggagttgtagta

SEQ ID NO: 125 - RNA, 21 nt, synthetic construct
  source 1..21: mol_type = other RNA
tacaactccagctccgtctat

SEQ ID NO: 126 - RNA, 23 nt, synthetic construct
  source 1..23: mol_type = other RNA
atagacggagctggagttgtagt

SEQ ID NO: 127 - RNA, 21 nt, synthetic construct
  source 1..21: mol_type = other RNA
acaactccagctccgtctatt

SEQ ID NO: 128 - RNA, 23 nt, synthetic construct
  source 1..23: mol_type = other RNA
aatagacggagctggagttgtag

SEQ ID NO: 129 - RNA, 21 nt, synthetic construct
  source 1..21: mol_type = other RNA
caactccagctccgtctatta

SEQ ID NO: 130 - RNA, 23 nt, synthetic construct
  source 1..23: mol_type = other RNA
taatagacggagctggagttgta

SEQ ID NO: 131 - RNA, 21 nt, synthetic construct
  source 1..21: mol_type = other RNA
aactccagctccgtctattca

SEQ ID NO: 132 - RNA, 23 nt, synthetic construct
  source 1..23: mol_type = other RNA
tgaatagacggagctggagttgt

SEQ ID NO: 133 - RNA, 21 nt, synthetic construct
  source 1..21: mol_type = other RNA
actccagctccgtctattcct

SEQ ID NO: 134 - RNA, 23 nt, synthetic construct
  source 1..23: mol_type = other RNA
aggaatagacggagctggagttg

SEQ ID NO: 135 - RNA, 21 nt, synthetic construct
  source 1..21: mol_type = other RNA
ctccagctccgtctattcctt

SEQ ID NO: 136 - RNA, 23 nt, synthetic construct
  source 1..23: mol_type = other RNA
aaggaatagacggagctggagtt

SEQ ID NO: 137 - RNA, 21 nt, synthetic construct
  source 1..21: mol_type = other RNA
tccaggcctgtgaagtgaaca

SEQ ID NO: 138 - RNA, 23 nt, synthetic construct
  source 1..23: mol_type = other RNA
tgttcacttcacaggcctggaag

SEQ ID NO: 139 - RNA, 21 nt, synthetic construct
  source 1..21: mol_type = other RNA
ccaggcctgtgaagtgaacct

SEQ ID NO: 140 - RNA, 23 nt, synthetic construct
  source 1..23: mol_type = other RNA
aggttcacttcacaggcctggaa

SEQ ID NO: 141 - RNA, 21 nt, synthetic construct
  source 1..21: mol_type = other RNA
caggcctgtgaagtgaaccta

SEQ ID NO: 142 - RNA, 23 nt, synthetic construct
  source 1..23: mol_type = other RNA
taggttcacttcacaggcctgga

SEQ ID NO: 143 - RNA, 21 nt, synthetic construct
  source 1..21: mol_type = other RNA
aggcctgtgaagtgaacctga

SEQ ID NO: 144 - RNA, 23 nt, synthetic construct
  source 1..23: mol_type = other RNA
tcaggttcacttcacaggcctgg

SEQ ID NO: 145 - RNA, 21 nt, synthetic construct
  source 1..21: mol_type = other RNA
ggcctgtgaagtgaacctgaa

SEQ ID NO: 146 - RNA, 23 nt, synthetic construct
  source 1..23: mol_type = other RNA
ttcaggttcacttcacaggcctg

SEQ ID NO: 147 - RNA, 21 nt, synthetic construct
  source 1..21: mol_type = other RNA
gcctgtgaagtgaacctgaca

SEQ ID NO: 148 - RNA, 23 nt, synthetic construct
  source 1..23: mol_type = other RNA
tgtcaggttcacttcacaggcct

SEQ ID NO: 149 - RNA, 21 nt, synthetic construct
  source 1..21: mol_type = other RNA
ctgtgaagtgaacctgacgct

SEQ ID NO: 150 - RNA, 23 nt, synthetic construct
  source 1..23: mol_type = other RNA
agcgtcaggttcacttcacaggc

SEQ ID NO: 151 - RNA, 21 nt, synthetic construct
  source 1..21: mol_type = other RNA
tgtgaagtgaacctgacgcta

SEQ ID NO: 152 - RNA, 23 nt, synthetic construct
  source 1..23: mol_type = other RNA
tagcgtcaggttcacttcacagg

SEQ ID NO: 153 - RNA, 21 nt, synthetic construct
  source 1..21: mol_type = other RNA
gtgaagtgaacctgacgctga

SEQ ID NO: 154 - RNA, 23 nt, synthetic construct
  source 1..23: mol_type = other RNA
tcagcgtcaggttcacttcacag

SEQ ID NO: 155 - RNA, 21 nt, synthetic construct
  source 1..21: mol_type = other RNA
atcgctgaccgctgggtgata

SEQ ID NO: 156 - RNA, 23 nt, synthetic construct
  source 1..23: mol_type = other RNA
tatcacccagcggtcagcgatga

SEQ ID NO: 157 - RNA, 21 nt, synthetic construct
  source 1..21: mol_type = other RNA
tcgctgaccgctgggtgataa

SEQ ID NO: 158 - RNA, 23 nt, synthetic construct
  source 1..23: mol_type = other RNA
ttatcacccagcggtcagcgatg

SEQ ID NO: 159 - RNA, 21 nt, synthetic construct
  source 1..21: mol_type = other RNA
cgctgaccgctgggtgataat

SEQ ID NO: 160 - RNA, 23 nt, synthetic construct
  source 1..23: mol_type = other RNA
attatcacccagcggtcagcgat

SEQ ID NO: 161 - RNA, 21 nt, synthetic construct
  source 1..21: mol_type = other RNA
gctgaccgctgggtgataaca

SEQ ID NO: 162 - RNA, 23 nt, synthetic construct
  source 1..23: mol_type = other RNA
tgttatcacccagcggtcagcga

SEQ ID NO: 163 - RNA, 21 nt, synthetic construct
  source 1..21: mol_type = other RNA
gaccgctgggtgataacagct

SEQ ID NO: 164 - RNA, 23 nt, synthetic construct
  source 1..23: mol_type = other RNA
agctgttatcacccagcggtcag

SEQ ID NO: 165 - RNA, 21 nt, synthetic construct
  source 1..21: mol_type = other RNA
accgctgggtgataacagcta

SEQ ID NO: 166 - RNA, 23 nt, synthetic construct
  source 1..23: mol_type = other RNA
tagctgttatcacccagcggtca

SEQ ID NO: 167 - RNA, 21 nt, synthetic construct
  source 1..21: mol_type = other RNA
tgctactctggtatttcctaa

SEQ ID NO: 168 - RNA, 23 nt, synthetic construct
  source 1..23: mol_type = other RNA
ttaggaaataccagagtagcacc

SEQ ID NO: 169 - RNA, 21 nt, synthetic construct
  source 1..21: mol_type = other RNA
gtgctactctggtatttccta

SEQ ID NO: 170 - RNA, 23 nt, synthetic construct
  source 1..23: mol_type = other RNA
taggaaataccagagtagcaccc

SEQ ID NO: 171 - RNA, 21 nt, synthetic construct
  source 1..21: mol_type = other RNA
ggtgctactctggtatttcct

SEQ ID NO: 172 - RNA, 23 nt, synthetic construct
  source 1..23: mol_type = other RNA
aggaaataccagagtagcacccc

SEQ ID NO: 173 - RNA, 21 nt, synthetic construct
  source 1..21: mol_type = other RNA
gggtgctactctggtatttca

SEQ ID NO: 174 - RNA, 23 nt, synthetic construct
  source 1..23: mol_type = other RNA
tgaaataccagagtagcaccccc

SEQ ID NO: 175 - RNA, 21 nt, synthetic construct
  source 1..21: mol_type = other RNA
ggggtgctactctggtattta

SEQ ID NO: 176 - RNA, 23 nt, synthetic construct
  source 1..23: mol_type = other RNA
taaataccagagtagcacccccg

SEQ ID NO: 177 - RNA, 21 nt, synthetic construct
  source 1..21: mol_type = other RNA
gggggtgctactctggtattt

SEQ ID NO: 178 - RNA, 23 nt, synthetic construct
  source 1..23: mol_type = other RNA
aaataccagagtagcacccccgc

SEQ ID NO: 179 - RNA, 21 nt, synthetic construct
  source 1..21: mol_type = other RNA
cgggggtgctactctggtatt

SEQ ID NO: 180 - RNA, 23 nt, synthetic construct
  source 1..23: mol_type = other RNA
aataccagagtagcacccccgcc

SEQ ID NO: 181 - RNA, 21 nt, synthetic construct
  source 1..21: mol_type = other RNA
gctactctggtatttcctagg

SEQ ID NO: 182 - RNA, 23 nt, synthetic construct
  source 1..23: mol_type = other RNA
cctaggaaataccagagtagcac

SEQ ID NO: 183 - RNA, 21 nt, synthetic construct
  source 1..21: mol_type = other RNA
ctactctggtatttcctaggg

SEQ ID NO: 184 - RNA, 23 nt, synthetic construct
  source 1..23: mol_type = other RNA
ccctaggaaataccagagtagca

SEQ ID NO: 185 - RNA, 21 nt, synthetic construct
  source 1..21: mol_type = other RNA
tactctggtatttcctagggt

SEQ ID NO: 186 - RNA, 23 nt, synthetic construct
  source 1..23: mol_type = other RNA
accctaggaaataccagagtagc

SEQ ID NO: 187 - RNA, 21 nt, synthetic construct
  source 1..21: mol_type = other RNA
tgctactctggtatttcctat

SEQ ID NO: 188 - RNA, 23 nt, synthetic construct
  source 1..23: mol_type = other RNA
ataggaaataccagagtagcacc